European Patent Application EP 4 477 673 A1, published December 18, 2024. Title: IMMUNOCONJUGATE AND USE THEREOF. Applicant: Jiangsu Hengrui Pharmaceuticals Co., Ltd. Application WO PCT/CN2023/075448, filed February 10, 2023. The sequence listing filed with the application follows.

SEQUENCE LISTING (109 sequences)

SEQ ID NO: 1 - protein, 288 aa, Homo sapiens
  source 1..288: note = PD-1
MQIPQAPWPVVWAVLQLGWRPGWFLDSPDRPWNPPTFSPALLVVTEGDNATFTCSFSNTSESFVLNWYRMSPSNQTDKLAAFPEDRSQPGQDCRFRVTQLPNGRDFHMSVVRARRNDSGTYLCGAISLAPKAQIKESLRAELRVTERRAEVPTAHPSPSPRPAGQFQTLVVGVVGGLLGSLVLLVWVLAVICSRAARGTIGARRTGQPLKEDPSAVPVFSVDYGELDFQWREKTPEPPVPCVPEQTEYATIVFPSGMGTSSPARRGSADGPRSAQPLRPEDGHCSWPL

SEQ ID NO: 2 - protein, 122 aa, synthetic construct
  source 1..122: note; note (original language) = A6 variable region
EVQLVESGGGLVQAGGSLRLSCAVSGRTFSSAAMGWFRQAPGKEREFVAAISWSFGSTYYADSVKGRFTISRDNAKNTVYLQMNSLKPEDTAVYYCAADPSIETMGGGWDYWGQGTQVTVSS

SEQ ID NO: 3 - protein, 116 aa, synthetic construct
  source 1..116: note; note (original language) = A17 variable region
EVQVVESGGGLVQPGGSLRLSCVASGLTFSDYSMSWYRQAPGKERELVAIISGSGVIAHYVDSVKGRFTISRDNAKSTVYLQMVSLKPEDRGVYYCRAVSDWDDYWGQGTQVTVSS

SEQ ID NO: 4 - protein, 5 aa, synthetic construct
  source 1..5: note = A6 CDR1
SAAMG

SEQ ID NO: 5 - protein, 16 aa, synthetic construct
  source 1..16: note = A6 CDR2
ISWSFGSTYYADSVKG

SEQ ID NO: 6 - protein, 13 aa, synthetic construct
  source 1..13: note = A6 CDR3
DPSIETMGGGWDY

SEQ ID NO: 7 - protein, 5 aa, synthetic construct
  source 1..5: note = A17 CDR1
DYSMS

SEQ ID NO: 8 - protein, 17 aa, synthetic construct
  source 1..17: note = A17 CDR1
IISGSGVIAHYVDSVKG

SEQ ID NO: 9 - protein, 7 aa, synthetic construct
  source 1..7: note = A17 CDR3
VSDWDDY

SEQ ID NO: 10 - protein, 229 aa, synthetic construct
  source 1..229: note = hIgG4
ESKYGPPCPPCPAPEFLGGPSVFLFPPKPKDTLMISRTPEVTCVVVDVSQEDPEVQFNWYVDGVEVHNAKTKPREEQFNSTYRVVSVLTVLHQDWLNGKEYKCKVSNKGLPSSIEKTISKAKGQPREPQVYTLPPSQEEMTKNQVSLTCLVKGFYPSDIAVEWESNGQPENNYKTTPPVLDSDGSFFLYSRLTVDKSRWQEGNVFSCSVMHEALHNHYTQKSLSLSLGK

SEQ ID NO: 11 - protein, 351 aa, synthetic construct
  source 1..351: note = A6_hIgG4
EVQLVESGGGLVQAGGSLRLSCAVSGRTFSSAAMGWFRQAPGKEREFVAAISWSFGSTYYADSVKGRFTISRDNAKNTVYLQMNSLKPEDTAVYYCAADPSIETMGGGWDYWGQGTQVTVSSESKYGPPCPPCPAPEFLGGPSVFLFPPKPKDTLMISRTPEVTCVVVDVSQEDPEVQFNWYVDGVEVHNAKTKPREEQFNSTYRVVSVLTVLHQDWLNGKEYKCKVSNKGLPSSIEKTISKAKGQPREPQVYTLPPSQEEMTKNQVSLTCLVKGFYPSDIAVEWESNGQPENNYKTTPPVLDSDGSFFLYSRLTVDKSRWQEGNVFSCSVMHEALHNHYTQKSLSLSLGK

SEQ ID NO: 12 - protein, 345 aa, synthetic construct
  source 1..345: note = A17_ hIgG4
EVQVVESGGGLVQPGGSLRLSCVASGLTFSDYSMSWYRQAPGKERELVAIISGSGVIAHYVDSVKGRFTISRDNAKSTVYLQMVSLKPEDRGVYYCRAVSDWDDYWGQGTQVTVSSESKYGPPCPPCPAPEFLGGPSVFLFPPKPKDTLMISRTPEVTCVVVDVSQEDPEVQFNWYVDGVEVHNAKTKPREEQFNSTYRVVSVLTVLHQDWLNGKEYKCKVSNKGLPSSIEKTISKAKGQPREPQVYTLPPSQEEMTKNQVSLTCLVKGFYPSDIAVEWESNGQPENNYKTTPPVLDSDGSFFLYSRLTVDKSRWQEGNVFSCSVMHEALHNHYTQKSLSLSLGK

SEQ ID NO: 13 - protein, 116 aa, synthetic construct
  source 1..116: note; note (original language) = A17h1 variable region
EVQLQESGGGLVQPGGSLRLSCTASGLTFSDYSMSWYRQAPGKGRELVAIISGSGVIAHYVDSVKGRFTISRDNSKNTVYLQMRSLTPEDRAVYYCRAVSDWDDYWGQGTQVTVSS

SEQ ID NO: 14 - protein, 116 aa, synthetic construct
  source 1..116: note; note (original language) = A17h2 variable region
EVQLVESGGGLVQPGGSLRLSCAASGLTFSDYSMSWVRQAPGKGLEWVAIISGSGVIAHYVDSVKGRFTISRDNSKNTVYLQMNSLRAEDTAVYYCRAVSDWDDYWGQGTQVTVSS

SEQ ID NO: 15 - protein, 116 aa, synthetic construct
  source 1..116: note; note (original language) = A17h3 variable region
EVQLVESGGGLVQPGGSLRLSCAASGLTFSDYSMSWVRQAPGKGLEWVAIISGSGVIAHYVDSVKGRFTISRDNSKNTVYLQMNSLRAEDTAVYYCRAVSDWDEYWGQGTQVTVSS

SEQ ID NO: 16 - protein, 122 aa, synthetic construct
  source 1..122: note; note (original language) = A6h1 variable region
EVQLLESGGGLVQAGGSLRLSCATSGRTFSSAAMGWFRQAPGKGLEWVAAISWSFGSTYYADSVKGRFTISRDNSKNTVYLQMNSLRPEDTAVYYCAADPSIETMGGGWDYWGQGTQVTVSS

SEQ ID NO: 17 - protein, 116 aa, synthetic construct
  source 1..116: note; note (original language) = A17m01 variable region
EVQLQESGGGLVQPGGSLRLSCTASGLTFSDYSMSWYRQAPGKGRELVAIISGSGVIAHYVDSVKGRFTISRDNAKNTVYLQMRSLTPEDRAVYYCRAVSDWDDYWGQGTQVTVSS

SEQ ID NO: 18 - protein, 116 aa, synthetic construct
  source 1..116: note; note (original language) = A17m02 variable region
EVQLQESGGGLVQPGGSLRLSCTASGLTFSDYSMSWYRQAPGKGRELVAIISGSGVITHYVDSVKGRFTISRDNSKNTVYLQMRSLTPEDRAVYYCRAVSDWDDYWGQGTQVTVSS

SEQ ID NO: 19 - protein, 116 aa, synthetic construct
  source 1..116: note; note (original language) = A17m03 variable region
EVQLQESGGGLVQPGGSLRLSCTASGLTFSDYSMSWYRQAPGKGRELVAIISGSGGIAHYVDSVKGRFTISRDNSKNTVYLQMRSLTPEDRAVYYCRAVSDWDDYWGQGTQVTVSS

SEQ ID NO: 20 - protein, 116 aa, synthetic construct
  source 1..116: note; note (original language) = A17m04 variable region
EVQLQESGGGLVQPGGSLRLSCTASGLTFSDYSMSWYRQAPGKGRELVAIISGSGVSAHYVDSVKGRFTISRDNSKNTVYLQMRSLTPEDRAVYYCRAVSDWDDYWGQGTQVTVSS

SEQ ID NO: 21 - protein, 116 aa, synthetic construct
  source 1..116: note; note (original language) = A17m05 variable region
EVQLQESGGGLVQPGGSLRLSCTASGLTFSDYSMSWYRQAPGKGRELVAIISGSGVIAHYVDSVKGRFTISRDNSKNTVYLQMRSLTPEDRAVYYCRAVSDWEDYWGQGTQVTVSS

SEQ ID NO: 22 - protein, 116 aa, synthetic construct
  source 1..116: note; note (original language) = A17m06 variable region
EVQLQESGGGLVQPGGSLRLSCTASGLTFSDYSMSWYRQAPGKGRELVAIISGSGVIAHYVDSVKGRFTISRDNSKNTVYLQMRSLTPEDRAVYYCRAVSDWDEYWGQGTQVTVSS

SEQ ID NO: 23 - protein, 116 aa, synthetic construct
  source 1..116: note; note (original language) = A17m07 variable region
EVQLQESGGGLVQPGGSLRLSCTASGLTFSDYSMSWYRQAPGKGRELVAIISGSGVIAHYVDSVKGRFTISRDNAKNTVYLQMRSLTPEDRAVYYCRAVSDWEDYWGQGTQVTVSS

SEQ ID NO: 24 - protein, 116 aa, synthetic construct
  source 1..116: note; note (original language) = A17m08 variable region
EVQLQESGGGLVQPGGSLRLSCTASGLTFSDYSMSWYRQAPGKGRELVAIISGSGVIAHYVDSVKGRFTISRDNAKNTVYLQMRSLTPEDRAVYYCRAVSDWDEYWGQGTQVTVSS

SEQ ID NO: 25 - protein, 116 aa, synthetic construct
  source 1..116: note; note (original language) = A17m09 variable region
EVQLQESGGGLVQPGGSLRLSCTASGLTFSDYSMSWYRQAPGKGRELVAIISGSGVITHYVDSVKGRFTISRDNAKNTVYLQMRSLTPEDRAVYYCRAVSDWEDYWGQGTQVTVSS

SEQ ID NO: 26 - protein, 116 aa, synthetic construct
  source 1..116: note; note (original language) = A17m10 variable region
EVQLQESGGGLVQPGGSLRLSCTASGLTFSDYSMSWYRQAPGKGRELVAIISGSGVITHYVDSVKGRFTISRDNAKNTVYLQMRSLTPEDRAVYYCRAVSDWDEYWGQGTQVTVSS

SEQ ID NO: 27 - protein, 116 aa, synthetic construct
  source 1..116: note; note (original language) = A17m11 variable region
EVQLQESGGGLVQPGGSLRLSCTASGLTFSDYSMSWYRQAPGKGRELVAIISGSGGIAHYVDSVKGRFTISRDNAKNTVYLQMRSLTPEDRAVYYCRAVSDWEDYWGQGTQVTVSS

SEQ ID NO: 28 - protein, 116 aa, synthetic construct
  source 1..116: note; note (original language) = A17m12 variable region
EVQLQESGGGLVQPGGSLRLSCTASGLTFSDYSMSWYRQAPGKGRELVAIISGSGGIAHYVDSVKGRFTISRDNAKNTVYLQMRSLTPEDRAVYYCRAVSDWDEYWGQGTQVTVSS

SEQ ID NO: 29 - protein, 116 aa, synthetic construct
  source 1..116: note; note (original language) = A17m13 variable region
EVQLQESGGGLVQPGGSLRLSCTASGLTFSDYSMSWYRQAPGKGRELVAIISGSGVSAHYVDSVKGRFTISRDNAKNTVYLQMRSLTPEDRAVYYCRAVSDWEDYWGQGTQVTVSS

SEQ ID NO: 30 - protein, 116 aa, synthetic construct
  source 1..116: note; note (original language) = A17m14 variable region
EVQLQESGGGLVQPGGSLRLSCTASGLTFSDYSMSWYRQAPGKGRELVAIISGSGVSAHYVDSVKGRFTISRDNAKNTVYLQMRSLTPEDRAVYYCRAVSDWDEYWGQGTQVTVSS

SEQ ID NO: 31 - protein, 116 aa, synthetic construct
  source 1..116: note; note (original language) = A17m15 variable region
EVQLQESGGGLVQPGGSLRLSCTASGLTFSDYSMSWYRQAPGKGRELVAIISGSGGITHYVDSVKGRFTISRDNAKNTVYLQMRSLTPEDRAVYYCRAVSDWEDYWGQGTQVTVSS

SEQ ID NO: 32 - protein, 116 aa, synthetic construct
  source 1..116: note; note (original language) = A17m0901 variable region
EVQLVESGGGLVQPGGSLRLSCAASGFTFSDYSMSWYRQAPGKGRELVAIISGSGVITHYVDSVKGRFTISRDNAKNTLYLQMRSLRAEDTAVYYCRAVSDWEDYWGQGTQVTVSS

SEQ ID NO: 33 - protein, 116 aa, synthetic construct
  source 1..116: note; note (original language) = A17m0902 variable region
EVQLVESGGGLVQPGGSLRLSCAASGLTFSDYSMSWYRQAPGKGRELVAIISGSGVITHYVDSVKGRFTISRDNAKNTLYLQMRSLRAEDTAVYYCRAVSDWEDYWGQGTQVTVSS

SEQ ID NO: 34 - protein, 116 aa, synthetic construct
  source 1..116: note; note (original language) = A17m0903 variable region
EVQLVESGGGLVQPGGSLRLSCAASGLTFSDYSMSWYRQAPGKGRELVAIISGSGVITHYVDSVKGRFTISRDNAKNTVYLQMRSLRAEDTAVYYCRAVSDWEDYWGQGTQVTVSS

SEQ ID NO: 35 - protein, 116 aa, synthetic construct
  source 1..116: note; note (original language) = A17m0905 variable region
EVQLVESGGGLVQPGGSLRLSCAASGLTFSDYSMSWYRQAPGKGRELVAIISGSGVITHYVDSVKGRFTISRDNAKNTVYLQMRSLRAEDRAVYYCRAVSDWEDYWGQGTQVTVSS

SEQ ID NO: 36 - protein, 17 aa, synthetic construct
  VARIANT 7: note; note (original language) = X is selected from the group consisting of V and G
  VARIANT 8: note; note (original language) = X is selected from the group consisting of I and S
  VARIANT 9: note; note (original language) = X is selected from the group consisting of T and A
IISGSGXXXHYVDSVKG

SEQ ID NO: 37 - protein, 7 aa, synthetic construct
  VARIANT 5: note; note (original language) = X is selected from the group consisting of D and E
  VARIANT 6: note; note (original language) = X is selected from the group consisting of D and E
VSDWXXY

SEQ ID NO: 38 - protein, 17 aa, synthetic construct
  source 1..17: note = CDR2
IISGSGVITHYVDSVKG

SEQ ID NO: 39 - protein, 17 aa, synthetic construct
  source 1..17: note = CDR2
IISGSGGIAHYVDSVKG

SEQ ID NO: 40 - protein, 17 aa, synthetic construct
  source 1..17: note = CDR2
IISGSGVSAHYVDSVKG

SEQ ID NO: 41 - protein, 7 aa, synthetic construct
  source 1..7: note = CDR3
VSDWEDY

SEQ ID NO: 42 - protein, 7 aa, synthetic construct
  source 1..7: note = CDR3
VSDWDEY

SEQ ID NO: 43 - protein, 495 aa, synthetic construct
  source 1..495: note; note (original language) = The Knob chain of A-V91T
EVQLQESGGGLVQPGGSLRLSCTASGLTFSDYSMSWYRQAPGKGRELVAIISGSGVIAHYVDSVKGRFTISRDNSKNTVYLQMRSLTPEDRAVYYCRAVSDWDDYWGQGTQVTVSSEPKSSDKTHTCPPCPAPEAAGGPSVFLFPPKPKDTLMISRTPEVTCVVVDVSHEDPEVKFNWYVDGVEVHNAKTKPREEQYNSTYRVVSVLTVLHQDWLNGKEYKCKVSNKALGAPIEKTISKAKGQPREPQVYTLPPCRDELTKNQVSLWCLVKGFYPSDIAVEWESNGQPENNYKTTPPVLDSDGSFFLYSKLTVDKSRWQQGNVFSCSVMHEALHNHYTQKSLSLSPGGGGGSGGGGSGGGGSAPASSSTKKTQLQLEHLLLDLQMILNGINNYKNPKLTEMLTAKFYMPKKATELKHLQCLEEELKPLEEVLNLAQSKNFHLRPRDLISNINTIVLELKGSETTFMCEYADETATIVEFLNRWITFAQSIISTLT

SEQ ID NO: 44 - protein, 346 aa, synthetic construct
  source 1..346: note; note (original language) = The Hole chain of A-V91T
EVQLQESGGGLVQPGGSLRLSCTASGLTFSDYSMSWYRQAPGKGRELVAIISGSGVIAHYVDSVKGRFTISRDNSKNTVYLQMRSLTPEDRAVYYCRAVSDWDDYWGQGTQVTVSSEPKSSDKTHTCPPCPAPEAAGGPSVFLFPPKPKDTLMISRTPEVTCVVVDVSHEDPEVKFNWYVDGVEVHNAKTKPREEQYNSTYRVVSVLTVLHQDWLNGKEYKCKVSNKALGAPIEKTISKAKGQPREPQVCTLPPSRDELTKNQVSLSCAVKGFYPSDIAVEWESNGQPENNYKTTPPVLDSDGSFFLVSKLTVDKSRWQQGNVFSCSVMHEALHNRFTQKSLSLSP

SEQ ID NO: 45 - protein, 621 aa, synthetic construct
  source 1..621: note; note (original language) = The Knob chain of B-V91T
EVQLQESGGGLVQPGGSLRLSCTASGLTFSDYSMSWYRQAPGKGRELVAIISGSGVIAHYVDSVKGRFTISRDNSKNTVYLQMRSLTPEDRAVYYCRAVSDWDDYWGQGTQVTVSSGGGGSGGGGSEVQLQESGGGLVQPGGSLRLSCTASGLTFSDYSMSWYRQAPGKGRELVAIISGSGVIAHYVDSVKGRFTISRDNSKNTVYLQMRSLTPEDRAVYYCRAVSDWDDYWGQGTQVTVSSEPKSSDKTHTCPPCPAPEAAGGPSVFLFPPKPKDTLMISRTPEVTCVVVDVSHEDPEVKFNWYVDGVEVHNAKTKPREEQYNSTYRVVSVLTVLHQDWLNGKEYKCKVSNKALGAPIEKTISKAKGQPREPQVYTLPPCRDELTKNQVSLWCLVKGFYPSDIAVEWESNGQPENNYKTTPPVLDSDGSFFLYSKLTVDKSRWQQGNVFSCSVMHEALHNHYTQKSLSLSPGGGGGSGGGGSGGGGSAPASSSTKKTQLQLEHLLLDLQMILNGINNYKNPKLTEMLTAKFYMPKKATELKHLQCLEEELKPLEEVLNLAQSKNFHLRPRDLISNINTIVLELKGSETTFMCEYADETATIVEFLNRWITFAQSIISTLT

SEQ ID NO: 46 - protein, 472 aa, synthetic construct
  source 1..472: note; note (original language) = The Hole chain of B-V91T
EVQLQESGGGLVQPGGSLRLSCTASGLTFSDYSMSWYRQAPGKGRELVAIISGSGVIAHYVDSVKGRFTISRDNSKNTVYLQMRSLTPEDRAVYYCRAVSDWDDYWGQGTQVTVSSGGGGSGGGGSEVQLQESGGGLVQPGGSLRLSCTASGLTFSDYSMSWYRQAPGKGRELVAIISGSGVIAHYVDSVKGRFTISRDNSKNTVYLQMRSLTPEDRAVYYCRAVSDWDDYWGQGTQVTVSSEPKSSDKTHTCPPCPAPEAAGGPSVFLFPPKPKDTLMISRTPEVTCVVVDVSHEDPEVKFNWYVDGVEVHNAKTKPREEQYNSTYRVVSVLTVLHQDWLNGKEYKCKVSNKALGAPIEKTISKAKGQPREPQVCTLPPSRDELTKNQVSLSCAVKGFYPSDIAVEWESNGQPENNYKTTPPVLDSDGSFFLVSKLTVDKSRWQQGNVFSCSVMHEALHNRFTQKSLSLSP

SEQ ID NO: 47 - protein, 597 aa, synthetic construct
  source 1..597: note; note (original language) = The Knob chain of C-V91T
QVQLVQSGVEVKKPGASVKVSCKASGYTFTNYYMYWVRQAPGQGLEWMGGINPSNGGTNFNEKFKNRVTLTTDSSTTTAYMELKSLQFDDTAVYYCARRDYRFDMGFDYWGQGTTVTVSSASTKGPSVFPLAPSSKSTSGGTAALGCLVKDYFPEPVTVSWNSGALTSGVHTFPAVLQSSGLYSLSSVVTVPSSSLGTQTYICNVNHKPSNTKVDKKVEPKSCDKTHTCPPCPAPEAAGGPSVFLFPPKPKDTLMISRTPEVTCVVVDVSHEDPEVKFNWYVDGVEVHNAKTKPREEQYNSTYRVVSVLTVLHQDWLNGKEYKCKVSNKALGAPIEKTISKAKGQPREPQVYTLPPCRDELTKNQVSLWCLVKGFYPSDIAVEWESNGQPENNYKTTPPVLDSDGSFFLYSKLTVDKSRWQQGNVFSCSVMHEALHNHYTQKSLSLSPGGGGGSGGGGSGGGGSAPASSSTKKTQLQLEHLLLDLQMILNGINNYKNPKLTEMLTAKFYMPKKATELKHLQCLEEELKPLEEVLNLAQSKNFHLRPRDLISNINTIVLELKGSETTFMCEYADETATIVEFLNRWITFAQSIISTLT

SEQ ID NO: 48 - protein, 218 aa, synthetic construct
  source 1..218: note; note (original language) = The light chain of C-V91T
EIVLTQSPATLSLSPGERATLSCRASKGVSTSGYSYLHWYQQKPGQAPRLLIYLASYLESGVPARFSGSGSGTDFTLTISSLEPEDFAVYYCQHSRDLPLTFGGGTKVEIKRTVAAPSVFIFPPSDEQLKSGTASVVCLLNNFYPREAKVQWKVDNALQSGNSQESVTEQDSKDSTYSLSSTLTLSKADYEKHKVYACEVTHQGLSSPVTKSFNRGEC

SEQ ID NO: 49 - protein, 723 aa, synthetic construct
  source 1..723: note; note (original language) = The Knob chain of E-V91T
EVQLQESGGGLVQPGGSLRLSCTASGLTFSDYSMSWYRQAPGKGRELVAIISGSGVIAHYVDSVKGRFTISRDNSKNTVYLQMRSLTPEDRAVYYCRAVSDWDDYWGQGTQVTVSSGGGGSGGGGSQVQLVQSGVEVKKPGASVKVSCKASGYTFTNYYMYWVRQAPGQGLEWMGGINPSNGGTNFNEKFKNRVTLTTDSSTTTAYMELKSLQFDDTAVYYCARRDYRFDMGFDYWGQGTTVTVSSASTKGPSVFPLAPSSKSTSGGTAALGCLVKDYFPEPVTVSWNSGALTSGVHTFPAVLQSSGLYSLSSVVTVPSSSLGTQTYICNVNHKPSNTKVDKKVEPKSCDKTHTCPPCPAPEAAGGPSVFLFPPKPKDTLMISRTPEVTCVVVDVSHEDPEVKFNWYVDGVEVHNAKTKPREEQYNSTYRVVSVLTVLHQDWLNGKEYKCKVSNKALGAPIEKTISKAKGQPREPQVYTLPPCRDELTKNQVSLWCLVKGFYPSDIAVEWESNGQPENNYKTTPPVLDSDGSFFLYSKLTVDKSRWQQGNVFSCSVMHEALHNHYTQKSLSLSPGGGGGSGGGGSGGGGSAPASSSTKKTQLQLEHLLLDLQMILNGINNYKNPKLTEMLTAKFYMPKKATELKHLQCLEEELKPLEEVLNLAQSKNFHLRPRDLISNINTIVLELKGSETTFMCEYADETATIVEFLNRWITFAQSIISTLT

SEQ ID NO: 50 - protein, 574 aa, synthetic construct
  source 1..574: note; note (original language) = The Hole chain of E-V91T
EVQLQESGGGLVQPGGSLRLSCTASGLTFSDYSMSWYRQAPGKGRELVAIISGSGVIAHYVDSVKGRFTISRDNSKNTVYLQMRSLTPEDRAVYYCRAVSDWDDYWGQGTQVTVSSGGGGSGGGGSQVQLVQSGVEVKKPGASVKVSCKASGYTFTNYYMYWVRQAPGQGLEWMGGINPSNGGTNFNEKFKNRVTLTTDSSTTTAYMELKSLQFDDTAVYYCARRDYRFDMGFDYWGQGTTVTVSSASTKGPSVFPLAPSSKSTSGGTAALGCLVKDYFPEPVTVSWNSGALTSGVHTFPAVLQSSGLYSLSSVVTVPSSSLGTQTYICNVNHKPSNTKVDKKVEPKSCDKTHTCPPCPAPEAAGGPSVFLFPPKPKDTLMISRTPEVTCVVVDVSHEDPEVKFNWYVDGVEVHNAKTKPREEQYNSTYRVVSVLTVLHQDWLNGKEYKCKVSNKALGAPIEKTISKAKGQPREPQVCTLPPSRDELTKNQVSLSCAVKGFYPSDIAVEWESNGQPENNYKTTPPVLDSDGSFFLVSKLTVDKSRWQQGNVFSCSVMHEALHNRFTQKSLSLSP

SEQ ID NO: 51 - protein, 369 aa, synthetic construct
  source 1..369: note; note (original language) = The Knob chain of F-V91T
APASSSTKKTQLQLEHLLLDLQMILNGINNYKNPKLTEMLTAKFYMPKKATELKHLQCLEEELKPLEEVLNLAQSKNFHLRPRDLISNINTIVLELKGSETTFMCEYADETATIVEFLNRWITFAQSIISTLTGGGGSEPKSSDKTHTCPPCPAPEAAGGPSVFLFPPKPKDTLMISRTPEVTCVVVDVSHEDPEVKFNWYVDGVEVHNAKTKPREEQYNSTYRVVSVLTVLHQDWLNGKEYKCKVSNKALGAPIEKTISKAKGQPREPQVYTLPPCRDELTKNQVSLWCLVKGFYPSDIAVEWESNGQPENNYKTTPPVLDSDGSFFLYSKLTVDKSRWQQGNVFSCSVMHEALHNHYTQKSLSLSPG

SEQ ID NO: 52 - protein, 218 aa, synthetic construct
  source 1..218: note; note (original language) = The Fab heavy chain of pembrolizumab
QVQLVQSGVEVKKPGASVKVSCKASGYTFTNYYMYWVRQAPGQGLEWMGGINPSNGGTNFNEKFKNRVTLTTDSSTTTAYMELKSLQFDDTAVYYCARRDYRFDMGFDYWGQGTTVTVSSASTKGPSVFPLAPSSKSTSGGTAALGCLVKDYFPEPVTVSWNSGALTSGVHTFPAVLQSSGLYSLSSVVTVPSSSLGTQTYICNVNHKPSNTKVDKKV

SEQ ID NO: 53 - protein, 218 aa, synthetic construct; identical to SEQ ID NO: 48
  source 1..218: note; note (original language) = The Fab light chain of pembrolizumab

SEQ ID NO: 54 - protein, 5 aa, synthetic construct
  source 1..5: note; note (original language) = The HCDR1 of pembrolizumab
NYYMY

SEQ ID NO: 55 - protein, 17 aa, synthetic construct
  source 1..17: note; note (original language) = The HCDR2 of pembrolizumab
GINPSNGGTNFNEKFKN

SEQ ID NO: 56 - protein, 11 aa, synthetic construct
  source 1..11: note; note (original language) = The HCDR3 of pembrolizumab
RDYRFDMGFDY

SEQ ID NO: 57 - protein, 15 aa, synthetic construct
  source 1..15: note; note (original language) = The LCDR1 of pembrolizumab
RASKGVSTSGYSYLH

SEQ ID NO: 58 - protein, 7 aa, synthetic construct
  source 1..7: note; note (original language) = The LCDR2 of pembrolizumab
LASYLES

SEQ ID NO: 59 - protein, 9 aa, synthetic construct
  source 1..9: note; note (original language) = The LCDR3 of pembrolizumab
QHSRDLPLT

SEQ ID NO: 60 - protein, 133 aa, synthetic construct
  source 1..133: note = IL-2v(V91T)
APASSSTKKTQLQLEHLLLDLQMILNGINNYKNPKLTEMLTAKFYMPKKATELKHLQCLEEELKPLEEVLNLAQSKNFHLRPRDLISNINTIVLELKGSETTFMCEYADETATIVEFLNRWITFAQSIISTLT

SEQ ID NO: 61 - protein, 133 aa, synthetic construct
  source 1..133: note; note (original language) = The IL-2 sequence in A-PC
APASSSTKKTQLQLEHLLLDLQMILQGISNYKNPKLTRMLTAKFYMPKKATELKHLQCLEEELKPLEEVLQGAQSKNFHLRPRDLISNINVIVLELKGSETTFMCEYADETATIVEFLNRWITFAQSIISTLT

SEQ ID NO: 62 - protein, 133 aa, synthetic construct
  source 1..133: note; note (original language) = The IL-2 sequence in A-V91T-02
APASSSTKKTQLQLEHLLLDLQMILQGISNYKNPKLTRMLTAKFYMPKKATELKHLQCLEEELKPLEEVLQGAQSKNFHLRPRDLISNINTIVLELKGSETTFMCEYADETATIVEFLNRWITFAQSIISTLT

SEQ ID NO: 63 - protein, 133 aa, synthetic construct
  source 1..133: note; note (original language) = The IL-2 sequence in A-D20A
APASSSTKKTQLQLEHLLLALQMILQGISNYKNPKLTRMLTAKFYMPKKATELKHLQCLEEELKPLEEVLQGAQSKNFHLRPRDLISNINVIVLELKGSETTFMCEYADETATIVEFLNRWITFAQSIISTLT

SEQ ID NO: 64 - protein, 133 aa, synthetic construct
  source 1..133: note; note (original language) = The IL-2 sequence in A-D20N
APASSSTKKTQLQLEHLLLNLQMILQGISNYKNPKLTRMLTAKFYMPKKATELKHLQCLEEELKPLEEVLQGAQSKNFHLRPRDLISNINVIVLELKGSETTFMCEYADETATIVEFLNRWITFAQSIISTLT

SEQ ID NO: 65 - protein, 133 aa, synthetic construct
  source 1..133: note; note (original language) = The IL-2 sequence in A-N88D
APASSSTKKTQLQLEHLLLDLQMILQGISNYKNPKLTRMLTAKFYMPKKATELKHLQCLEEELKPLEEVLQGAQSKNFHLRPRDLISDINVIVLELKGSETTFMCEYADETATIVEFLNRWITFAQSIISTLT

SEQ ID NO: 66 - protein, 133 aa, synthetic construct
  source 1..133: note; note (original language) = The IL-2 sequence in A-N88R
APASSSTKKTQLQLEHLLLDLQMILQGISNYKNPKLTRMLTAKFYMPKKATELKHLQCLEEELKPLEEVLQGAQSKNFHLRPRDLISRINVIVLELKGSETTFMCEYADETATIVEFLNRWITFAQSIISTLT

SEQ ID NO: 67 - protein, 133 aa, synthetic construct
  source 1..133: note; note (original language) = The IL-2 sequence in A-Q126D
APASSSTKKTQLQLEHLLLDLQMILQGISNYKNPKLTRMLTAKFYMPKKATELKHLQCLEEELKPLEEVLQGAQSKNFHLRPRDLISNINVIVLELKGSETTFMCEYADETATIVEFLNRWITFADSIISTLT

SEQ ID NO: 68 - protein, 133 aa, synthetic construct
  source 1..133: note; note (original language) = The IL-2 sequence in A-H16A/D84S
APASSSTKKTQLQLEALLLDLQMILQGISNYKNPKLTRMLTAKFYMPKKATELKHLQCLEEELKPLEEVLQGAQSKNFHLRPRSLISNINVIVLELKGSETTFMCEYADETATIVEFLNRWITFAQSIISTLT

SEQ ID NO: 69 - protein, 231 aa, synthetic construct
  source 1..231: note; note (original language) = The Knob chain of Fc (D356, L358)
EPKSSDKTHTCPPCPAPEAAGGPSVFLFPPKPKDTLMISRTPEVTCVVVDVSHEDPEVKFNWYVDGVEVHNAKTKPREEQYNSTYRVVSVLTVLHQDWLNGKEYKCKVSNKALPAPIEKTISKAKGQPREPQVYTLPPCRDELTKNQVSLWCLVKGFYPSDIAVEWESNGQPENNYKTTPPVLDSDGSFFLYSKLTVDKSRWQQGNVFSCSVMHEALHNHYTQKSLSLSPG

SEQ ID NO: 70 - protein, 230 aa, synthetic construct
  source 1..230: note; note (original language) = The Hole chain of Fc (D356, L358)
EPKSSDKTHTCPPCPAPEAAGGPSVFLFPPKPKDTLMISRTPEVTCVVVDVSHEDPEVKFNWYVDGVEVHNAKTKPREEQYNSTYRVVSVLTVLHQDWLNGKEYKCKVSNKALPAPIEKTISKAKGQPREPQVCTLPPSRDELTKNQVSLSCAVKGFYPSDIAVEWESNGQPENNYKTTPPVLDSDGSFFLVSKLTVDKSRWQQGNVFSCSVMHEALHNHYTQKSLSLSP

SEQ ID NO: 71 - protein, 231 aa, synthetic construct
  source 1..231: note; note (original language) = The Knob chain of Fc (E356, M358)
EPKSSDKTHTCPPCPAPEAAGGPSVFLFPPKPKDTLMISRTPEVTCVVVDVSHEDPEVKFNWYVDGVEVHNAKTKPREEQYNSTYRVVSVLTVLHQDWLNGKEYKCKVSNKALPAPIEKTISKAKGQPREPQVYTLPPCREEMTKNQVSLWCLVKGFYPSDIAVEWESNGQPENNYKTTPPVLDSDGSFFLYSKLTVDKSRWQQGNVFSCSVMHEALHNHYTQKSLSLSPG

SEQ ID NO: 72 - protein, 231 aa, synthetic construct
  source 1..231: note; note (original language) = The Hole chain of Fc (E356, M358)
EPKSSDKTHTCPPCPAPEAAGGPSVFLFPPKPKDTLMISRTPEVTCVVVDVSHEDPEVKFNWYVDGVEVHNAKTKPREEQYNSTYRVVSVLTVLHQDWLNGKEYKCKVSNKALPAPIEKTISKAKGQPREPQVCTLPPSREEMTKNQVSLSCAVKGFYPSDIAVEWESNGQPENNYKTTPPVLDSDGSFFLVSKLTVDKSRWQQGNVFSCSVMHEALHNHYTQKSLSLSPG

SEQ ID NO: 73 - protein, 495 aa, synthetic construct
  source 1..495: note; note (original language) = The Knob chain of A-D20A (D356, L358)
EVQLVESGGGLVQPGGSLRLSCAASGLTFSDYSMSWYRQAPGKGRELVAIISGSGVITHYVDSVKGRFTISRDNAKNTLYLQMRSLRAEDTAVYYCRAVSDWEDYWGQGTQVTVSSEPKSSDKTHTCPPCPAPEAAGGPSVFLFPPKPKDTLMISRTPEVTCVVVDVSHEDPEVKFNWYVDGVEVHNAKTKPREEQYNSTYRVVSVLTVLHQDWLNGKEYKCKVSNKALPAPIEKTISKAKGQPREPQVYTLPPCRDELTKNQVSLWCLVKGFYPSDIAVEWESNGQPENNYKTTPPVLDSDGSFFLYSKLTVDKSRWQQGNVFSCSVMHEALHNHYTQKSLSLSPGGGGGSGGGGSGGGGSAPASSSTKKTQLQLEHLLLALQMILQGISNYKNPKLTRMLTAKFYMPKKATELKHLQCLEEELKPLEEVLQGAQSKNFHLRPRDLISNINVIVLELKGSETTFMCEYADETATIVEFLNRWITFAQSIISTLT

SEQ ID NO: 74 - protein, 346 aa, synthetic construct
  source 1..346: note; note (original language) = The Hole chain of A-D20A (D356, L358)
EVQLVESGGGLVQPGGSLRLSCAASGLTFSDYSMSWYRQAPGKGRELVAIISGSGVITHYVDSVKGRFTISRDNAKNTLYLQMRSLRAEDTAVYYCRAVSDWEDYWGQGTQVTVSSEPKSSDKTHTCPPCPAPEAAGGPSVFLFPPKPKDTLMISRTPEVTCVVVDVSHEDPEVKFNWYVDGVEVHNAKTKPREEQYNSTYRVVSVLTVLHQDWLNGKEYKCKVSNKALPAPIEKTISKAKGQPREPQVCTLPPSRDELTKNQVSLSCAVKGFYPSDIAVEWESNGQPENNYKTTPPVLDSDGSFFLVSKLTVDKSRWQQGNVFSCSVMHEALHNRFTQKSLSLSP

SEQ ID NO: 75 - protein, 495 aa, synthetic construct
  source 1..495: note; note (original language) = The Knob chain of A-D20A (E356, M358)
EVQLVESGGGLVQPGGSLRLSCAASGLTFSDYSMSWYRQAPGKGRELVAIISGSGVITHYVDSVKGRFTISRDNAKNTLYLQMRSLRAEDTAVYYCRAVSDWEDYWGQGTQVTVSSEPKSSDKTHTCPPCPAPEAAGGPSVFLFPPKPKDTLMISRTPEVTCVVVDVSHEDPEVKFNWYVDGVEVHNAKTKPREEQYNSTYRVVSVLTVLHQDWLNGKEYKCKVSNKALPAPIEKTISKAKGQPREPQVYTLPPCREEMTKNQVSLWCLVKGFYPSDIAVEWESNGQPENNYKTTPPVLDSDGSFFLYSKLTVDKSRWQQGNVFSCSVMHEALHNHYTQKSLSLSPGGGGGSGGGGSGGGGSAPASSSTKKTQLQLEHLLLALQMILQGISNYKNPKLTRMLTAKFYMPKKATELKHLQCLEEELKPLEEVLQGAQSKNFHLRPRDLISNINVIVLELKGSETTFMCEYADETATIVEFLNRWITFAQSIISTLT

SEQ ID NO: 76 - protein, 347 aa, synthetic construct
  source 1..347: note; note (original language) = The Hole chain of A-D20A (E356, M358)
EVQLVESGGGLVQPGGSLRLSCAASGLTFSDYSMSWYRQAPGKGRELVAIISGSGVITHYVDSVKGRFTISRDNAKNTLYLQMRSLRAEDTAVYYCRAVSDWEDYWGQGTQVTVSSEPKSSDKTHTCPPCPAPEAAGGPSVFLFPPKPKDTLMISRTPEVTCVVVDVSHEDPEVKFNWYVDGVEVHNAKTKPREEQYNSTYRVVSVLTVLHQDWLNGKEYKCKVSNKALPAPIEKTISKAKGQPREPQVCTLPPSREEMTKNQVSLSCAVKGFYPSDIAVEWESNGQPENNYKTTPPVLDSDGSFFLVSKLTVDKSRWQQGNVFSCSVMHEALHNHYTQKSLSLSPG

SEQ ID NO: 77 - protein, 495 aa, synthetic construct
  source 1..495: note; note (original language) = The Knob chain of A-N88D (D356, L358)
EVQLVESGGGLVQPGGSLRLSCAASGLTFSDYSMSWYRQAPGKGRELVAIISGSGVITHYVDSVKGRFTISRDNAKNTLYLQMRSLRAEDTAVYYCRAVSDWEDYWGQGTQVTVSSEPKSSDKTHTCPPCPAPEAAGGPSVFLFPPKPKDTLMISRTPEVTCVVVDVSHEDPEVKFNWYVDGVEVHNAKTKPREEQYNSTYRVVSVLTVLHQDWLNGKEYKCKVSNKALPAPIEKTISKAKGQPREPQVYTLPPCRDELTKNQVSLWCLVKGFYPSDIAVEWESNGQPENNYKTTPPVLDSDGSFFLYSKLTVDKSRWQQGNVFSCSVMHEALHNHYTQKSLSLSPGGGGGSGGGGSGGGGSAPASSSTKKTQLQLEHLLLDLQMILQGISNYKNPKLTRMLTAKFYMPKKATELKHLQCLEEELKPLEEVLQGAQSKNFHLRPRDLISDINVIVLELKGSETTFMCEYADETATIVEFLNRWITFAQSIISTLT

SEQ ID NO: 78 - protein, 346 aa, synthetic construct
  source 1..346: note; note (original language) = The Hole chain of A-N88D (D356, L358)
EVQLVESGGGLVQPGGSLRLSCAASGLTFSDYSMSWYRQAPGKGRELVAIISGSGVITHYVDSVKGRFTISRDNAKNTLYLQMRSLRAEDTAVYYCRAVSDWEDYWGQGTQVTVSSEPKSSDKTHTCPPCPAPEAAGGPSVFLFPPKPKDTLMISRTPEVTCVVVDVSHEDPEVKFNWYVDGVEVHNAKTKPREEQYNSTYRVVSVLTVLHQDWLNGKEYKCKVSNKALPAPIEKTISKAKGQPREPQVCTLPPSRDELTKNQVSLSCAVKGFYPSDIAVEWESNGQPENNYKTTPPVLDSDGSFFLVSKLTVDKSRWQQGNVFSCSVMHEALHNHYTQKSLSLSP

SEQ ID NO: 79 - protein, 495 aa, synthetic construct
  source 1..495: note; note (original language) = The Knob chain of A-N88D (E356, M358)
EVQLVESGGGLVQPGGSLRLSCAASGLTFSDYSMSWYRQAPGKGRELVAIISGSGVITHYVDSVKGRFTISRDNAKNTLYLQMRSLRAEDTAVYYCRAVSDWEDYWGQGTQVTVSSEPKSSDKTHTCPPCPAPEAAGGPSVFLFPPKPKDTLMISRTPEVTCVVVDVSHEDPEVKFNWYVDGVEVHNAKTKPREEQYNSTYRVVSVLTVLHQDWLNGKEYKCKVSNKALPAPIEKTISKAKGQPREPQVYTLPPCREEMTKNQVSLWCLVKGFYPSDIAVEWESNGQPENNYKTTPPVLDSDGSFFLYSKLTVDKSRWQQGNVFSCSVMHEALHNHYTQKSLSLSPGGGGGSGGGGSGGGGSAPASSSTKKTQLQLEHLLLDLQMILQGISNYKNPKLTRMLTAKFYMPKKATELKHLQCLEEELKPLEEVLQGAQSKNFHLRPRDLISDINVIVLELKGSETTFMCEYADETATIVEFLNRWITFAQSIISTLT

SEQ ID NO: 80 - protein, 347 aa, synthetic construct; identical to SEQ ID NO: 76
  source 1..347: note; note (original language) = The Hole chain of A-N88D (E356, M358)

SEQ ID NO: 81 - protein, 595 aa, synthetic construct
  source 1..595: note; note (original language) = The Knob chain of IgG-PC
QVQLVQSGAEVKKPGASVKVSCKASGYTFTNSWIGWFRQAPGQGLEWIGDIYPGGGYTNYNEIFKGKATMTADTSTNTAYMELSSLRSEDTAVYYCSRGIPGYAMDYWGQGTLVTVSSASTKGPSVFPLAPSSKSTSGGTAALGCLVKDYFPEPVTVSWNSGALTSGVHTFPAVLQSSGLYSLSSVVTVPSSSLGTQTYICNVNHKPSNTKVDKKVEPKSCDKTHTCPPCPAPEAAGGPSVFLFPPKPKDTLMISRTPEVTCVVVDVSHEDPEVKFNWYVDGVEVHNAKTKPREEQYNSTYRVVSVLTVLHQDWLNGKEYKCKVSNKALGAPIEKTISKAKGQPREPQVYTLPPCRDELTKNQVSLWCLVKGFYPSDIAVEWESNGQPENNYKTTPPVLDSDGSFFLYSKLTVDKSRWQQGNVFSCSVMHEALHNHYTQKSLSLSPGGGGGSGGGGSGGGGSAPASSSTKKTQLQLEHLLLDLQMILQGISNYKNPKLTRMLTAKFYMPKKATELKHLQCLEEELKPLEEVLQGAQSKNFHLRPRDLISNINVIVLELKGSETTFMCEYADETATIVEFLNRWITFAQSIISTLT

SEQ ID NO: 82 - protein, 595 aa, synthetic construct
  source 1..595: note; note (original language) = The Knob chain of IgG-V91T
QVQLVQSGAEVKKPGASVKVSCKASGYTFTNSWIGWFRQAPGQGLEWIGDIYPGGGYTNYNEIFKGKATMTADTSTNTAYMELSSLRSEDTAVYYCSRGIPGYAMDYWGQGTLVTVSSASTKGPSVFPLAPSSKSTSGGTAALGCLVKDYFPEPVTVSWNSGALTSGVHTFPAVLQSSGLYSLSSVVTVPSSSLGTQTYICNVNHKPSNTKVDKKVEPKSCDKTHTCPPCPAPEAAGGPSVFLFPPKPKDTLMISRTPEVTCVVVDVSHEDPEVKFNWYVDGVEVHNAKTKPREEQYNSTYRVVSVLTVLHQDWLNGKEYKCKVSNKALGAPIEKTISKAKGQPREPQVYTLPPCRDELTKNQVSLWCLVKGFYPSDIAVEWESNGQPENNYKTTPPVLDSDGSFFLYSKLTVDKSRWQQGNVFSCSVMHEALHNHYTQKSLSLSPGGGGGSGGGGSGGGGSAPASSSTKKTQLQLEHLLLDLQMILNGINNYKNPKLTEMLTAKFYMPKKATELKHLQCLEEELKPLEEVLNLAQSKNFHLRPRDLISNINTIVLELKGSETTFMCEYADETATIVEFLNRWITFAQSIISTLT

SEQ ID NO: 83 - protein, 595 aa, synthetic construct
  source 1..595: note; note (original language) = The Knob chain of IgG-N88D
QVQLVQSGAEVKKPGASVKVSCKASGYTFTNSWIGWFRQAPGQGLEWIGDIYPGGGYTNYNEIFKGKATMTADTSTNTAYMELSSLRSEDTAVYYCSRGIPGYAMDYWGQGTLVTVSSASTKGPSVFPLAPSSKSTSGGTAALGCLVKDYFPEPVTVSWNSGALTSGVHTFPAVLQSSGLYSLSSVVTVPSSSLGTQTYICNVNHKPSNTKVDKKVEPKSCDKTHTCPPCPAPEAAGGPSVFLFPPKPKDTLMISRTPEVTCVVVDVSHEDPEVKFNWYVDGVEVHNAKTKPREEQYNSTYRVVSVLTVLHQDWLNGKEYKCKVSNKALGAPIEKTISKAKGQPREPQVYTLPPCRDELTKNQVSLWCLVKGFYPSDIAVEWESNGQPENNYKTTPPVLDSDGSFFLYSKLTVDKSRWQQGNVFSCSVMHEALHNHYTQKSLSLSPGGGGGSGGGGSGGGGSAPASSSTKKTQLQLEHLLLDLQMILQGISNYKNPKLTRMLTAKFYMPKKATELKHLQCLEEELKPLEEVLQGAQSKNFHLRPRDLISDINVIVLELKGSETTFMCEYADETATIVEFLNRWITFAQSIISTLT

SEQ ID NO: 84 - protein, 595 aa, synthetic construct
  source 1..595: note; note (original language) = The Knob chain of IgG-D20A
QVQLVQSGAEVKKPGASVKVSCKASGYTFTNSWIGWFRQAPGQGLEWIGDIYPGGGYTNYNEIFKGKATMTADTSTNTAYMELSSLRSEDTAVYYCSRGIPGYAMDYWGQGTLVTVSSASTKGPSVFPLAPSSKSTSGGTAALGCLVKDYFPEPVTVSWNSGALTSGVHTFPAVLQSSGLYSLSSVVTVPSSSLGTQTYICNVNHKPSNTKVDKKVEPKSCDKTHTCPPCPAPEAAGGPSVFLFPPKPKDTLMISRTPEVTCVVVDVSHEDPEVKFNWYVDGVEVHNAKTKPREEQYNSTYRVVSVLTVLHQDWLNGKEYKCKVSNKALGAPIEKTISKAKGQPREPQVYTLPPCRDELTKNQVSLWCLVKGFYPSDIAVEWESNGQPENNYKTTPPVLDSDGSFFLYSKLTVDKSRWQQGNVFSCSVMHEALHNHYTQKSLSLSPGGGGGSGGGGSGGGGSAPASSSTKKTQLQLEHLLLALQMILQGISNYKNPKLTRMLTAKFYMPKKATELKHLQCLEEELKPLEEVLQGAQSKNFHLRPRDLISNINVIVLELKGSETTFMCEYADETATIVEFLNRWITFAQSIISTLT

SEQ ID NO: 85 - protein, 446 aa, synthetic construct
  source 1..446: note; note (original language) = The Hole chain of IgG-PC, IgG-V91T, IgG-D20A, or IgG-N88D
QVQLVQSGAEVKKPGASVKVSCKASGYTFTNSWIGWFRQAPGQGLEWIGDIYPGGGYTNYNEIFKGKATMTADTSTNTAYMELSSLRSEDTAVYYCSRGIPGYAMDYWGQGTLVTVSSASTKGPSVFPLAPSSKSTSGGTAALGCLVKDYFPEPVTVSWNSGALTSGVHTFPAVLQSSGLYSLSSVVTVPSSSLGTQTYICNVNHKPSNTKVDKKVEPKSCDKTHTCPPCPAPEAAGGPSVFLFPPKPKDTLMISRTPEVTCVVVDVSHEDPEVKFNWYVDGVEVHNAKTKPREEQYNSTYRVVSVLTVLHQDWLNGKEYKCKVSNKALGAPIEKTISKAKGQPREPQVCTLPPSRDELTKNQVSLSCAVKGFYPSDIAVEWESNGQPENNYKTTPPVLDSDGSFFLVSKLTVDKSRWQQGNVFSCSVMHEALHNRFTQKSLSLSP

SEQ ID NO: 86 - protein, 220 aa, synthetic construct
  source 1..220: note; note (original language) = The light chain of IgG-PC, IgG-V91T, IgG-D20A, or IgG-N88D
DIQMTQSPSSLSASVGDRVTMSCKSSQSLLNSGDQKNYLTWYQQKPGKAPKLLIYWASTGESGVPSRFSGSGSGTDFTFTISSLQPEDIATYYCQNDYSYPWTFGQGTKVEIKRTVAAPSVFIFPPSDEQLKSGTASVVCLLNNFYPREAKVQWKVDNALQSGNSQESVTEQDSKDSTYSLSSTLTLSKADYEKHKVYACEVTHQGLSSPVTKSFNRGEC

SEQ ID NO: 87 - protein, 133 aa, synthetic construct [sequence omitted]

SEQ ID NO: 88 - protein, 116 aa, synthetic construct
  source 1..116: note = A17m0902M08
EVQLVESGGGLVQPGGSLRLSCAASGLTFSDYSMSWYRQAPGKGRELVAIISGSGVITHYVDSVKGRFTISRDNAKNTLYLQMRSLRAEDTAVYYCRAVSDWQDYWGQGTQVTVSS

SEQ ID NO: 89 - protein, 116 aa, synthetic construct
  source 1..116: note = A17m0902M15
EVQLVESGGGLVQPGGSLRLSCAASGLTFSDYSMSWYRQAPGKGRELVAIISGSGGITHYVDSVKGRFTISRDNAKNTLYLQMRSLRAEDTAVYYCRAVSDWEDYWGQGTQVTVSS

SEQ ID NO: 90 - protein, 116 aa, synthetic construct
  source 1..116: note = A17m0902M26
EVQLVESGGGLVQPGGSLRLSCAASGLTFSSYSMSWYRQAPGKGRELVAIISGSGGITHYVDSVKGRFTISRDNAKNTLYLQMRSLRAEDTAVYYCRAVSDWEDYWGQGTQVTVSS

SEQ ID NO: 91 - protein, 116 aa, synthetic construct
  source 1..116: note = A17m0902M27
EVQLVESGGGLVQPGGSLRLSCAASGLTFSSYSMSWYRQAPGKGRELVAIISGSGGITHYVDSVKGRFTISRDNAKNTLYLQMRSLRAEDTAVYYCRAVSDWQDYWGQGTQVTVSS

SEQ ID NO: 92 - protein, 116 aa, synthetic construct
  source 1..116: note = A17m0902M28
EVQLVESGGGLVQPGGSLRLSCAASGLTFSSYSMSWYRQAPGKGRELVAIISGSGGITHYADSVKGRFTISRDNAKNTLYLQMRSLRAEDTAVYYCRAVSDWQDYWGQGTQVTVSS

SEQ ID NO: 93 - protein, 5 aa, synthetic construct
  source 1..5: note = CDR1
SYSMS

SEQ ID NO: 94 - protein, 17 aa, synthetic construct
  source 1..17: note = CDR2
IISGSGGITHYVDSVKG

SEQ ID NO: 95 - protein, 17 aa, synthetic construct
  source 1..17: note = CDR2
IISGSGGITHYADSVKG

SEQ ID NO: 96 - protein, 7 aa, synthetic construct
  source 1..7: note = CDR3
VSDWQDY

SEQ ID NO: 97 - protein, 5 aa, synthetic construct
  source 1..5: note = CDR1
  VARIANT 1: note; note (original language) = X is selected from the group consisting of D and S
XYSMS

SEQ ID NO: 98 - protein, 17 aa, synthetic construct
  source 1..17: note = CDR2
  VARIANT 7: note; note (original language) = X is selected from the group consisting of V and G
  VARIANT 12: note; note (original language) = X is selected from the group consisting of V and A
IISGSGXITHYXDSVKG

SEQ ID NO: 99 - protein, 7 aa, synthetic construct
  source 1..7: note = CDR3
  VARIANT 5: note; note (original language) = X is selected from the group consisting of Q and E
VSDWXDY

SEQ ID NO: 100 - protein, 17 aa, synthetic construct
  source 1..17: note = CDR2
  VARIANT 7: note; note (original language) = X is selected from the group consisting of V and G
  VARIANT 8: note; note (original language) = X is selected from the group consisting of I and S
  VARIANT 9: note; note (original language) = X is selected from the group consisting of T and A
  VARIANT 12: note; note (original language) = X is selected from the group consisting of V and A
IISGSGXXXHYXDSVKG

SEQ ID NO: 101 - protein, 7 aa, synthetic construct
  source 1..7: note = CDR3
  VARIANT 5: note; note (original language) = X is selected from the group consisting of Q, D, and E
  VARIANT 6: note; note (original language) = X is selected from the group consisting of D and E
VSDWXXY

SEQ ID NO: 102 - protein, 495 aa, synthetic construct
  source 1..495: note; note (original language) = The Knob chain of A-N88D-M08
EVQLVESGGGLVQPGGSLRLSCAASGLTFSDYSMSWYRQAPGKGRELVAIISGSGVITHYVDSVKGRFTISRDNAKNTLYLQMRSLRAEDTAVYYCRAVSDWQDYWGQGTQVTVSSEPKSSDKTHTCPPCPAPEAAGGPSVFLFPPKPKDTLMISRTPEVTCVVVDVSHEDPEVKFNWYVDGVEVHNAKTKPREEQYNSTYRVVSVLTVLHQDWLNGKEYKCKVSNKALPAPIEKTISKAKGQPREPQVYTLPPCREEMTKNQVSLWCLVKGFYPSDIAVEWESNGQPENNYKTTPPVLDSDGSFFLYSKLTVDKSRWQQGNVFSCSVMHEALHNHYTQKSLSLSPGGGGGSGGGGSGGGGSAPASSSTKKTQLQLEHLLLDLQMILQGISNYKNPKLTRMLTAKFYMPKKATELKHLQCLEEELKPLEEVLQGAQSKNFHLRPRDLISDINVIVLELKGSETTFMCEYADETATIVEFLNRWITFAQSIISTLT

SEQ ID NO: 103 - protein, 347 aa, synthetic construct
  source 1..347: note; note (original language) = The Hole chain of A-N88D-M08
EVQLVESGGGLVQPGGSLRLSCAASGLTFSDYSMSWYRQAPGKGRELVAIISGSGVITHYVDSVKGRFTISRDNAKNTLYLQMRSLRAEDTAVYYCRAVSDWQDYWGQGTQVTVSSEPKSSDKTHTCPPCPAPEAAGGPSVFLFPPKPKDTLMISRTPEVTCVVVDVSHEDPEVKFNWYVDGVEVHNAKTKPREEQYNSTYRVVSVLTVLHQDWLNGKEYKCKVSNKALPAPIEKTISKAKGQPREPQVCTLPPSREEMTKNQVSLSCAVKGFYPSDIAVEWESNGQPENNYKTTPPVLDSDGSFFLVSKLTVDKSRWQQGNVFSCSVMHEALHNHYTQKSLSLSPG

SEQ ID NO: 104 - protein, 15 aa, synthetic construct
  source 1..15: note; note (original language) = Linker 1
GGGGSGGGGSGGGGS

SEQ ID NO: 105 - protein, 10 aa, synthetic construct
  source 1..10: note; note (original language) = Linker 2
GGGGSGGGGS

SEQ ID NO: 106 - protein, 5 aa, synthetic construct
  source 1..5: note; note (original language) = Linker 1
GGGGS

SEQ ID NO: 107 - protein, 100 aa, synthetic construct
  source 1..100: note; note (original language) = Linker
  REGION 1..100: note; note (original language) = A maximum of 19 GGNGT copies can be deleted
GGNGTGGNGTGGNGTGGNGTGGNGTGGNGTGGNGTGGNGTGGNGTGGNGTGGNGTGGNGTGGNGTGGNGTGGNGTGGNGTGGNGTGGNGTGGNGTGGNGT

SEQ ID NO: 108 - protein, 100 aa, synthetic construct
  source 1..100: note; note (original language) = Linker
  REGION 1..100: note; note (original language) = A maximum of 19 YGNGT copies can be deleted
YGNGTYGNGTYGNGTYGNGTYGNGTYGNGTYGNGTYGNGTYGNGTYGNGTYGNGTYGNGTYGNGTYGNGTYGNGTYGNGTYGNGTYGNGTYGNGTYGNGT

SEQ ID NO: 109 - protein, 100 aa, synthetic construct
  source 1..100: note; note (original language) = Linker
  REGION 1..100: note; note (original language) = A maximum of 19 EPKSS copies can be deleted
EPKSSEPKSSEPKSSEPKSSEPKSSEPKSSEPKSSEPKSSEPKSSEPKSSEPKSSEPKSSEPKSSEPKSSEPKSSEPKSSEPKSSEPKSSEPKSSEPKSS